European Patent Application EP 4 736 958 A2, published May 6, 2026. Title: ANTI-5T4 ANTIBODIES AND USES THEREOF. Applicant: Concept to Medicine Biotech Co., Ltd. Application WO. The sequence listing filed with the application follows.

SEQUENCE LISTING (267 sequences)

SEQ ID NO: 1 - protein, 115 aa, synthetic construct
EVQLQQSGPELVKPGASVKISCKASGYAFSSSWMNWVKQRPGKGLEWIGRIYREDGHTNYNGKFKGKATLTADKSSTTAYMQLTSLTSEDSAVYFCANGGAMDYWGQGTSVTVSS

SEQ ID NO: 2 - protein, 107 aa, synthetic construct
DIQMTQSTSSLSASLGDRVTISCRASQDISNYLNWYQQKPDGTVKLLIYYTSRLHSGVPSRFSGSGSGTDYSLTISNLEQEDIATYFCQQDNTLPWTFGGGTKLEIK

SEQ ID NO: 3 - protein, 122 aa, synthetic construct
EVKLVESGGGLVQPGGSLSLSCAASGFTFTDYYMSWVRQPPGKALEWLGFIRNKGNGYTTENSASVKGRFTISRDNSQSILYLQMNALRAEDSATYYCARYRGNPHYAMDYWGQGTSVTVSS

SEQ ID NO: 4 - protein, 111 aa, synthetic construct
DIVLTQFPASLAVSLGQRATISCRASESVEFYGTSFLQWYQQKPGQPPKLLIYGASNVESGVPARFSGSGSGTDFSLSIHPVEEDDIAMYFCQQSRKVPSTFGGGTKLEIK

SEQ ID NO: 5 - protein, 118 aa, synthetic construct
DVQLQESGPGLVKPSQSLSLTCSVTGYSITSGYYWNWIRQFPGNKLEWMGYINSDGSNNYNPSLKNRISITRDTSKNQFFLKLNSVTTEDTATYYCAREEYDYWFAYWGQGTLVTVSA

SEQ ID NO: 6 - protein, 107 aa, synthetic construct
DIVMTQSQKFMSTSVGDRVSVTCKASQNVGTNVAWYQQKPGQSPKALIYSASNRYSGVPDRFTGSGFGTDFTLTISNVQSEDLTEYFCQQYNSYPYTFGGGTNLEIK

SEQ ID NO: 7 - protein, 120 aa, synthetic construct
DVQLVESGGGLVQPGGSRKLSCTASGFTFSNFGMHWVRQAPETGLEWVAYISSGSSTFYYADSVKGRFTISRDNPKNTLFLQMTSLRSEDTAMYFCARSPAYYRYGLDYWGQGTTLTVSS

SEQ ID NO: 8 - protein, 111 aa, synthetic construct
DIVLTQSPASLAVSLGQRATISCRASQSVSSSTFSYMHWYQQKPGQPPKLLIKSSSNLESGVPARFSGSGSGTDFTLNIHPVEEEDTATYYCQHSWEIPYTFGGGTKLEIK

SEQ ID NO: 9 - protein, 121 aa, synthetic construct
EVQLVESGGGLVKPGGSLKLSCAASGFTFSDYGMHWVRQAPEKGLEWVAYISSGTSTIYYTDTVKGRFTISRDNAKNTLFLQMTSLRSEDTAMYYCARGGDGYYRSTMDYWGQGISVTVSS

SEQ ID NO: 10 - protein, 111 aa, synthetic construct
DIVLTQSPASLAVSLGQRATISCRASQSVSSSSYSYMHWYQQKPGQPPKLLIKSASNLASGVPARFSGSGSGTDFTLNIHPVEEEDSATYYCQHSWEVPRTFGGGTKLEIK

SEQ ID NO: 11 - protein, 120 aa, synthetic construct
DVQLVESGGGLVQPGGSRKLSCAASGFTFSSFGMHWVRQAPEKGLEWVAYISSGSSTIYYADTVKGRFTISRDNPKNTLFLQMTSLRSEDTAMYYCARNRAYHREAMDYWGQGTSVTVSS

SEQ ID NO: 12 - protein, 111 aa, synthetic construct
DIVLTQSPASLTVSLGQRATISCRASQSVSSSSYNYMHWYQQKPGQPPKLLIKSASNLESGVPARFSGSGSGTDFTLNIHPVEEEDTATYYCQHSWEIPYTFGGGTKLEIK

SEQ ID NO: 13 - protein, 116 aa, synthetic construct
QVLLQQSGAEVARPGASVKLSCKASGYTFTSYGLNWLRQRTGQGLEWIGEIYPRSENTHYNEKFKGKATLTADKSSSTAYMELRSLTSEDSAVYFCARGDWDFDHWGQGTTLTVSS

SEQ ID NO: 14 - protein, 106 aa, synthetic construct
EILLTQSPAIIPASPGEKVTITCSASSSVSYMNWYQQKPGSSPKIWIYGISNLASGVPARFSGSGSGTFFSFTINSMEAEDVATYYCQQRSSYPRTFGGGTKLEIK

SEQ ID NO: 15 - protein, 116 aa, synthetic construct
QVQLQQPGTELVKPGASVKLSCKASDYTFTSYWMHWVKQRPEQGLEWIGNINPSNGNTNYNEKFKNKATLTVDKSSSTAYMQLSSLTFEDSAVYYCARGGWDFDYWGQGTTLTVSS

SEQ ID NO: 16 - protein, 107 aa, synthetic construct
QVVLTQSPAIMSASPGEKVTMTCSASSSVRYMHWYQQRSGTSPKRWIYDTSKLTSGVPARFSGSGSGTSYSLTISSMEAEDAATYYCQLWTSKPPWTFGGGTKLEIR

SEQ ID NO: 17 - protein, 116 aa, synthetic construct
QVQLQQPGTELVKPGASVKLSCKASGYTFTSYWMHWVKQRPEQGLEWIGNINPSNGNTNYNENFKSQATLTVDKSSSTAYMQLSSLTSEDSAVYYCARGGWDFDYWGQGTTLTVSS

SEQ ID NO: 18 - protein, 107 aa, synthetic construct
QVVLTQSPAIMSASPGEKVTMTCSASSSVRYIHWYQQRSGTSPKRWIYDTSKLTSGVPVRFSGSGSGTSYSLTISSMEAEDAATYYCQQWTSKPPWTFGGGTKLEIR

SEQ ID NO: 19 - protein, 116 aa, synthetic construct
QVQLQQPGTELVKPGASVKLSCKASGYTFTSYWMHWVKQRPEQGLEWIGNINPSNGNTNYNERFKSKATLTVDKSSSTAYMQLSSLTSEDSTVYYCARGGWDFDYWGQGTTLTVSS

SEQ ID NO: 20 - protein, 107 aa, synthetic construct
QVVLTQSPAIMSASPGEKVTMTCSASSSVRYIHWYQQRSGTSPKRWIYDTSKLTSGVPVRFSGSGSGTSFSLTISSMEAEDAATYYCQQWTSKPPWTFGGGTKLEIK

SEQ ID NO: 21 - protein, 116 aa, synthetic construct
QVQLQQSGAELMKPGASVKLSCKATGYTFTGYWIEWVKQRPGQGLEWIGETLPGRGSTNYNEKFKGKATFTADTSSNIVYMQLSSLTIEDSAIYYCARGRRDFDYWGQGTTLTVSS

SEQ ID NO: 22 - protein, 107 aa, synthetic construct
DIQMTQTTSSLSASLGDEVTISCSASQGINNYLNWYQQKPDGTVKLLIYYTSSLHSGVPSRFSGSGSGTDYSLTIINLEPEDIATYYCQQFSKLPFTFGSGTKLEIR

SEQ ID NO: 23 - protein, 118 aa, synthetic construct
DVQLHESGPGLVKPSQSLSLTCSVTGYSITNNYYWNWIRQFPGNNLEWMGYITYDGSNNYNPSLKNRISVTRDTSKNQFFLKLSSVTTEDTATYYCTRGGGQLRFDYWGQGTTLTVSS

SEQ ID NO: 24 - protein, 107 aa, synthetic construct
SIVMTQTPKFLIVSAGDRVTITCKASQSVSNEVTWYQQKPGQSPKMLIYYASNRYTGVPDRFTGSGYGTDFTFTINTVQAEDLAIYFCQQDYSSPWTFGGGTKLEIK

SEQ ID NO: 25 - protein, 118 aa, synthetic construct
QVQLQQPGAELVKPGASVKMSCKASGYTFTSYWITWVKQRPGQGLERIGDIYPGSGTINYNEKFKSKATLTVDTSSSTAYMQLSSLTSEDSAVYCCARSDGNYYFDYWGQGTTLKVSS

SEQ ID NO: 26 - protein, 106 aa, synthetic construct
QIVLSQSPAILSASPGEKVTMTCRASSSVNYMHWYQQKPGSSPKPWIYATSNLASGVPVRFSGSGSGTSYSLTISRVEAEDAATYYCQQWSSNPPTFGGGTKLEIK

SEQ ID NO: 27 - protein, 119 aa, synthetic construct
DVQFQESGPGLVKPSQSLSLTCSVTGYSITSSYYWNWIRQFPGDKLEWMGYISYDGSNNYNPSLKNRISITRDTSKKQFFLKLNSVTTEDTATYYCARSWDGGYAMDNWGQGTSVTVSS

SEQ ID NO: 28 - protein, 107 aa, synthetic construct
SIVMTQTPKFLLVSAGDRVTITCKASQSVSNDVAWYQQKPGQSPKLLIYFASNRYTGVPDRFTGSGYGTVFTFTISTVQADDLAVYFCQQDYTSPWTFGGGTRLEIK

SEQ ID NO: 29 - protein, 121 aa, synthetic construct
EVQLQQSGAELVKPGASVKLSCTASGFNIKDTYMHWVKQRPEQGLEWIGRIDPANGHTIFASKFQGKATITADTSSNTAYMQLSSLTSGDTAVYYCGLFTMVVVPWYFDVWGTGTTVTVSS

SEQ ID NO: 30 - protein, 107 aa, synthetic construct
DIVMTQSHKFMSTSVGDRVSITCKASQDVSTAVAWYQQKPGQSPKLLIYWASTRHTGVPDRFTGSGSGTDYTLTISSVQAEDLALYYCQQHYSSPLTFGAGTKLELK

SEQ ID NO: 31 - protein, 121 aa, synthetic construct
QVQLQQSGAELVRPGSSVRISCKASGYAFSNYWMNWVKQRPGQGLEWIGQIYPGDGDTNYNGKFKNKATLTTDKSSSTAYMQLSSLTSEDSAVYFCARHYDYPYYYAMDYWGQGTSVTVSS

SEQ ID NO: 32 - protein, 107 aa, synthetic construct
DIQMTQSPSSLSASLGERVSLTCRASQDIGIALTWLQQEPDGTIKRLIYATSSLDSGVPKRFSGSRSGSDYTLTISSLESEDFVDYYCLQYIISPYTFGGGTKLEIK

SEQ ID NO: 33 - protein, 123 aa, synthetic construct
EVQLQQSGPELVKPGASVKISCKASGYTFTDYYMNWVKQSHGKSLEWIGDINPYSGGATNNQKFKGKATLTVDKSSSTAYIELRSLTSEDSAVYFCARGSIYYDSTANYFDYWGQGTTLTVSS

SEQ ID NO: 34 - protein, 107 aa, synthetic construct
DIQMTQSPASLSASVGETVTITCRASENIYSYLAWYQQKQGKSPQLLVYNAKSLTEGVPSRFSGSRSGTQFSLKINSLQPEDFGSYYCQHHYVTPWTFGGGTKLEIK

SEQ ID NO: 35 - protein, 118 aa, synthetic construct
QVQLQQSGPEVVKPGASVKISCKASGYTFTDYYMNWVKQSRGKSLEWIGDINPNNGGTNYNQKFKGKATLTVDKSSSTAYMELRSLTSEDSAVYYCAKEGPPGAMDYWGQGTSVTVSS

SEQ ID NO: 36 - protein, 107 aa, synthetic construct
NIVMTQTPKFLLVSAGDRVTITCKASQSVSNHVAWYQQKPGQSPKLLIYYVSNRSIGVPDRFTGSGYGTDFTFTISTVQAEDLAVYFCQQVYSSPFTFGGGTRLEMK

SEQ ID NO: 37 - protein, 118 aa, synthetic construct
QVQLQQSGPELVKPGASVKISCKASGYTFTAYYVNWVKQSHGKSLEWIGDINPNNGGTNYNQKFKGKATLTVDMSSSTAYMELRSLTSEDSAVYYCAKEGPPGAMDYWGQGTSVTVSS

SEQ ID NO: 38 - protein, 107 aa, synthetic construct
SIVLTQTPKFLLVSAGDRVPITCKASQSVSNNVAWYQQKPGQSPKLLIYYASNPYTGVPDRFTGSGYGTDFTFTITTVQAEDLAVYFCQQVYSSPFTFGGGTKLEMK

SEQ ID NO: 39 - protein, 118 aa, synthetic construct
QVQLQQSGPEVVNPGASVKISCKASGYTFTDYYMNWVKQSRGKSLEWIGDINPNNGGTNYNQKFKDKATLTVDKSSNTAYMELRSLTSENSAVYYCAKEGPPGAMDYWGQGTSVTVSS

SEQ ID NO: 40 - protein, 107 aa, synthetic construct
NIVMTQTPKFLLVSAGDRVTITCKASQSVSNHVAWYQQKPGQSPKLLIYYVSNRYIGVPDRFTGSGYGTDFTFTISTVQAEDLAVYFCQQVYSSPFTFGGGTRLEMK

SEQ ID NO: 41 - protein, 5 aa, synthetic construct
SSWMN

SEQ ID NO: 42 - protein, 17 aa, synthetic construct
RIYREDGHTNYNGKFKG

SEQ ID NO: 43 - protein, 6 aa, synthetic construct
GGAMDY

SEQ ID NO: 44 - protein, 11 aa, synthetic construct
RASQDISNYLN

SEQ ID NO: 45 - protein, 7 aa, synthetic construct
YTSRLHS

SEQ ID NO: 46 - protein, 9 aa, synthetic construct
QQDNTLPWT

SEQ ID NO: 47 - protein, 17 aa, synthetic construct
RIYREDAHTNYNGKFKG

SEQ ID NO: 48 - protein, 17 aa, synthetic construct
RIYREDGHTNYNAKFKG

SEQ ID NO: 49 - protein, 17 aa, synthetic construct
RIYREDGHTNYNQKFKG

SEQ ID NO: 50 - protein, 17 aa, synthetic construct
RIYREEGHTNYNQKFKG

SEQ ID NO: 51 - protein, 17 aa, synthetic construct
RIYREEGHTNYNEKFKG

SEQ ID NO: 52 - protein, 17 aa, synthetic construct
RIYRESGHTNYNQKFKG

SEQ ID NO: 53 - protein, 17 aa, synthetic construct
RIYRESGHTNYNEKFKG

SEQ ID NO: 54 - protein, 5 aa, synthetic construct
DYYMS

SEQ ID NO: 55 - protein, 19 aa, synthetic construct
FIRNKGNGYTTENSASVKG

SEQ ID NO: 56 - protein, 11 aa, synthetic construct
YRGNPHYAMDY

SEQ ID NO: 57 - protein, 15 aa, synthetic construct
RASESVEFYGTSFLQ

SEQ ID NO: 58 - protein, 7 aa, synthetic construct
GASNVES

SEQ ID NO: 59 - protein, 9 aa, synthetic construct
QQSRKVPST

SEQ ID NO: 60 - protein, 19 aa, synthetic construct
FIRNKGNAYTTEYSASVKG

SEQ ID NO: 61 - protein, 19 aa, synthetic construct
FIRNKGNTYTTEYSASVKG

SEQ ID NO: 62 - protein, 19 aa, synthetic construct
FIRNKGNAYTTENAASVKG

SEQ ID NO: 63 - protein, 19 aa, synthetic construct
FIRNKGNTYTTENAASVKG

SEQ ID NO: 64 - protein, 6 aa, synthetic construct
SGYYWN

SEQ ID NO: 65 - protein, 16 aa, synthetic construct
YINSDGSNNYNPSLKN

SEQ ID NO: 66 - protein, 9 aa, synthetic construct
EEYDYWFAY

SEQ ID NO: 67 - protein, 11 aa, synthetic construct
KASQNVGTNVA

SEQ ID NO: 68 - protein, 7 aa, synthetic construct
SASNRYS

SEQ ID NO: 69 - protein, 9 aa, synthetic construct
QQYNSYPYT

SEQ ID NO: 70 - protein, 5 aa, synthetic construct
NFGMH

SEQ ID NO: 71 - protein, 17 aa, synthetic construct
YISSGSSTFYYADSVKG

SEQ ID NO: 72 - protein, 11 aa, synthetic construct
SPAYYRYGLDY

SEQ ID NO: 73 - protein, 15 aa, synthetic construct
RASQSVSSSTFSYMH

SEQ ID NO: 74 - protein, 7 aa, synthetic construct
SSSNLES

SEQ ID NO: 75 - protein, 9 aa, synthetic construct
QHSWEIPYT

SEQ ID NO: 76 - protein, 17 aa, synthetic construct
YISSGSSTFYYADAVKG

SEQ ID NO: 77 - protein, 5 aa, synthetic construct
DYGMH

SEQ ID NO: 78 - protein, 17 aa, synthetic construct
YISSGTSTIYYTDTVKG

SEQ ID NO: 79 - protein, 12 aa, synthetic construct
GGDGYYRSTMDY

SEQ ID NO: 80 - protein, 15 aa, synthetic construct
RASQSVSSSSYSYMH

SEQ ID NO: 81 - protein, 7 aa, synthetic construct
SASNLAS

SEQ ID NO: 82 - protein, 9 aa, synthetic construct
QHSWEVPRT

SEQ ID NO: 83 - protein, 5 aa, synthetic construct
SFGMH

SEQ ID NO: 84 - protein, 17 aa, synthetic construct
YISSGSSTIYYADTVKG

SEQ ID NO: 85 - protein, 11 aa, synthetic construct
NRAYHREAMDY

SEQ ID NO: 86 - protein, 15 aa, synthetic construct
RASQSVSSSSYNYMH

SEQ ID NO: 87 - protein, 7 aa, synthetic construct
SASNLES

SEQ ID NO: 88 - protein, 9 aa, synthetic construct
QHSWEIPYT

SEQ ID NO: 89 - protein, 5 aa, synthetic construct
SYGLN

SEQ ID NO: 90 - protein, 17 aa, synthetic construct
EIYPRSENTHYNEKFKG

SEQ ID NO: 91 - protein, 7 aa, synthetic construct
GDWDFDH

SEQ ID NO: 92 - protein, 10 aa, synthetic construct
SASSSVSYMN

SEQ ID NO: 93 - protein, 7 aa, synthetic construct
GISNLAS

SEQ ID NO: 94 - protein, 9 aa, synthetic construct
QQRSSYPRT

SEQ ID NO: 95 - protein, 5 aa, synthetic construct
SYWMH

SEQ ID NO: 96 - protein, 17 aa, synthetic construct
NINPSNGNTNYNEKFKN

SEQ ID NO: 97 - protein, 7 aa, synthetic construct
GGWDFDY

SEQ ID NO: 98 - protein, 10 aa, synthetic construct
SASSSVRYMH

SEQ ID NO: 99 - protein, 7 aa, synthetic construct
DTSKLTS

SEQ ID NO: 100 - protein, 10 aa, synthetic construct
QLWTSKPPWT

SEQ ID NO: 101 - protein, 17 aa, synthetic construct
NINPSNANTNYNEKFKN

SEQ ID NO: 102 - protein, 17 aa, synthetic construct
NINPSNQNTNYNEKFKN

SEQ ID NO: 103 - protein, 17 aa, synthetic construct
NINPSNENTNYNEKFKN

SEQ ID NO: 104 - protein, 17 aa, synthetic construct
NINPSQGNTNYNEKFKN

SEQ ID NO: 105 - protein, 5 aa, synthetic construct
SYWMH

SEQ ID NO: 106 - protein, 17 aa, synthetic construct
NINPSNGNTNYNENFKS

SEQ ID NO: 107 - protein, 7 aa, synthetic construct
GGWDFDY

SEQ ID NO: 108 - protein, 10 aa, synthetic construct
SASSSVRYIH

SEQ ID NO: 109 - protein, 7 aa, synthetic construct
DTSKLTS

SEQ ID NO: 110 - protein, 10 aa, synthetic construct
QQWTSKPPWT

SEQ ID NO: 111 - protein, 5 aa, synthetic construct
SYWMH

SEQ ID NO: 112 - protein, 17 aa, synthetic construct
NINPSNGNTNYNERFKS

SEQ ID NO: 113 - protein, 7 aa, synthetic construct
GGWDFDY

SEQ ID NO: 114 - protein, 10 aa, synthetic construct
SASSSVRYIH

SEQ ID NO: 115 - protein, 7 aa, synthetic construct
DTSKLTS

SEQ ID NO: 116 - protein, 10 aa, synthetic construct
QQWTSKPPWT

SEQ ID NO: 117 - protein, 5 aa, synthetic construct
GYWIE

SEQ ID NO: 118 - protein, 17 aa, synthetic construct
ETLPGRGSTNYNEKFKG

SEQ ID NO: 119 - protein, 7 aa, synthetic construct
GRRDFDY

SEQ ID NO: 120 - protein, 11 aa, synthetic construct
SASQGINNYLN

SEQ ID NO: 121 - protein, 7 aa, synthetic construct
YTSSLHS

SEQ ID NO: 122 - protein, 9 aa, synthetic construct
QQFSKLPFT

SEQ ID NO: 123 - protein, 6 aa, synthetic construct
NNYYWN

SEQ ID NO: 124 - protein, 16 aa, synthetic construct
YITYDGSNNYNPSLKN

SEQ ID NO: 125 - protein, 9 aa, synthetic construct
GGGQLRFDY

SEQ ID NO: 126 - protein, 11 aa, synthetic construct
KASQSVSNEVT

SEQ ID NO: 127 - protein, 7 aa, synthetic construct
YASNRYT

SEQ ID NO: 128 - protein, 9 aa, synthetic construct
QQDYSSPWT

SEQ ID NO: 129 - protein, 16 aa, synthetic construct
YITYDASNNYNPSLKN

SEQ ID NO: 130 - protein, 5 aa, synthetic construct
SYWIT

SEQ ID NO: 131 - protein, 17 aa, synthetic construct
DIYPGSGTINYNEKFKS

SEQ ID NO: 132 - protein, 9 aa, synthetic construct
SDGNYYFDY

SEQ ID NO: 133 - protein, 10 aa, synthetic construct
RASSSVNYMH

SEQ ID NO: 134 - protein, 7 aa, synthetic construct
ATSNLAS

SEQ ID NO: 135 - protein, 9 aa, synthetic construct
QQWSSNPPT

SEQ ID NO: 136 - protein, 6 aa, synthetic construct
SSYYWN

SEQ ID NO: 137 - protein, 16 aa, synthetic construct
YISYDGSNNYNPSLKN

SEQ ID NO: 138 - protein, 10 aa, synthetic construct
SWDGGYAMDN

SEQ ID NO: 139 - protein, 11 aa, synthetic construct
KASQSVSNDVA

SEQ ID NO: 140 - protein, 7 aa, synthetic construct
FASNRYT

SEQ ID NO: 141 - protein, 9 aa, synthetic construct
QQDYTSPWT

SEQ ID NO: 142 - protein, 5 aa, synthetic construct
DTYMH

SEQ ID NO: 143 - protein, 17 aa, synthetic construct
RIDPANGHTIFASKFQG

SEQ ID NO: 144 - protein, 12 aa, synthetic construct
FTMVVVPWYFDV

SEQ ID NO: 145 - protein, 11 aa, synthetic construct
KASQDVSTAVA

SEQ ID NO: 146 - protein, 7 aa, synthetic construct
WASTRHT

SEQ ID NO: 147 - protein, 9 aa, synthetic construct
QQHYSSPLT

SEQ ID NO: 148 - protein, 5 aa, synthetic construct
NYWMN

SEQ ID NO: 149 - protein, 17 aa, synthetic construct
QIYPGDGDTNYNGKFKN

SEQ ID NO: 150 - protein, 12 aa, synthetic construct
HYDYPYYYAMDY

SEQ ID NO: 151 - protein, 11 aa, synthetic construct
RASQDIGIALT

SEQ ID NO: 152 - protein, 7 aa, synthetic construct
ATSSLDS

SEQ ID NO: 153 - protein, 9 aa, synthetic construct
LQYIISPYT

SEQ ID NO: 154 - protein, 5 aa, synthetic construct
DYYMN

SEQ ID NO: 155 - protein, 17 aa, synthetic construct
DINPYSGGATNNQKFKG

SEQ ID NO: 156 - protein, 14 aa, synthetic construct
GSIYYDSTANYFDY

SEQ ID NO: 157 - protein, 11 aa, synthetic construct
RASENIYSYLA

SEQ ID NO: 158 - protein, 7 aa, synthetic construct
NAKSLTE

SEQ ID NO: 159 - protein, 9 aa, synthetic construct
QHHYVTPWT

SEQ ID NO: 160 - protein, 5 aa, synthetic construct
DYYMN

SEQ ID NO: 161 - protein, 17 aa, synthetic construct
DINPNNGGTNYNQKFKG

SEQ ID NO: 162 - protein, 9 aa, synthetic construct
EGPPGAMDY

SEQ ID NO: 163 - protein, 11 aa, synthetic construct
KASQSVSNHVA

SEQ ID NO: 164 - protein, 7 aa, synthetic construct
YVSNRSI

SEQ ID NO: 165 - protein, 9 aa, synthetic construct
QQVYSSPFT

SEQ ID NO: 166 - protein, 17 aa, synthetic construct
DINPNQGGTNYNQKFKG

SEQ ID NO: 167 - protein, 5 aa, synthetic construct
AYYVN

SEQ ID NO: 168 - protein, 17 aa, synthetic construct
DINPNNGGTNYNQKFKG

SEQ ID NO: 169 - protein, 9 aa, synthetic construct
EGPPGAMDY

SEQ ID NO: 170 - protein, 11 aa, synthetic construct
KASQSVSNNVA

SEQ ID NO: 171 - protein, 7 aa, synthetic construct
YASNPYT

SEQ ID NO: 172 - protein, 9 aa, synthetic construct
QQVYSSPFT

SEQ ID NO: 173 - protein, 17 aa, synthetic construct
DINPNQGGTNYNQKFKG

SEQ ID NO: 174 - protein, 5 aa, synthetic construct
DYYMN

SEQ ID NO: 175 - protein, 17 aa, synthetic construct
DINPNNGGTNYNQKFKD

SEQ ID NO: 176 - protein, 9 aa, synthetic construct
EGPPGAMDY

SEQ ID NO: 177 - protein, 11 aa, synthetic construct
KASQSVSNHVA

SEQ ID NO: 178 - protein, 7 aa, synthetic construct
YVSNRYI

SEQ ID NO: 179 - protein, 9 aa, synthetic construct
QQVYSSPFT

SEQ ID NO: 180 - protein, 17 aa, synthetic construct
DINPNQGGTNYNQKFKD

SEQ ID NO: 181 - protein, 115 aa, synthetic construct
EVQLVQSGAEVKKPGATVKISCKVSGYAFSSSWMNWVQQAPGKGLEWMGRIYREDGHTNYNGKFKGRVTITADTSTDTAYMELSSLRSEDTAVYYCATGGAMDYWGQGTLVTVSS

SEQ ID NO: 182 - protein, 115 aa, synthetic construct
EVQLVQSGAEVKKPGATVKISCKVSGYAFSSSWMNWVQQAPGKGLEWIGRIYREDGHTNYNGKFKGRVTITADTSTDTAYMELSSLRSEDTAVYFCANGGAMDYWGQGTLVTVSS

SEQ ID NO: 183 - protein, 115 aa, synthetic construct
EVQLVQSGAEVKKPGATVKISCKVSGYAFSSSWMNWVKQAPGKGLEWIGRIYREDGHTNYNGKFKGRATITADTSTTTAYMELSSLRSEDTAVYFCANGGAMDYWGQGTLVTVSS

SEQ ID NO: 184 - protein, 115 aa, synthetic construct
EVQLVQSGAEVKKPGATVKISCKASGYAFSSSWMNWVKQAPGKGLEWIGRIYREDGHTNYNGKFKGRATITADTSTTTAYMELSSLRSEDSAVYFCANGGAMDYWGQGTLVTVSS

SEQ ID NO: 185 - protein, 107 aa, synthetic construct
DIQMTQSPSSLSASVGDRVTITCRASQDISNYLNWYQQKPGKAPKLLIYYTSRLHSGVPSRFSGSGSGTDFTFTISSLQPEDIATYYCQQDNTLPWTFGGGTKLEIK

SEQ ID NO: 186 - protein, 107 aa, synthetic construct
DIQMTQSPSSLSASVGDRVTITCRASQDISNYLNWYQQKPGKAPKLLIYYTSRLHSGVPSRFSGSGSGTDYTFTISSLQPEDIATYFCQQDNTLPWTFGGGTKLEIK

SEQ ID NO: 187 - protein, 107 aa, synthetic construct
DIQMTQSPSSLSASVGDRVTISCRASQDISNYLNWYQQKPGKAVKLLIYYTSRLHSGVPSRFSGSGSGTDFTFTISSLQPEDIATYFCQQDNTLPWTFGGGTKLEIK

SEQ ID NO: 188 - protein, 107 aa, synthetic construct
DIQMTQSPSSLSASVGDRVTISCRASQDISNYLNWYQQKPGKTVKLLIYYTSRLHSGVPSRFSGSGSGTDYTFTISSLQPEDIATYFCQQDNTLPWTFGGGTKLEIK

SEQ ID NO: 189 - protein, 115 aa, synthetic construct
QVQLVQSGAEVKKPGSSVKVSCKASGGTFSSSWMNWVRQAPGQGLEWMGRIYREDGHTNYNGKFKGRATITADKSTSTAYMELSSLRSEDTAVYYCARGGAMDYWGQGTTVTVSS

SEQ ID NO: 190 - protein, 115 aa, synthetic construct
QVQLVQSGAEVKKPGSSVKVSCKASGGTFSSSWMNWVKQAPGQGLEWIGRIYREDGHTNYNGKFKGKATLTADKSTSTAYMELSSLRSEDTAVYFCANGGAMDYWGQGTTVTVSS

SEQ ID NO: 191 - protein, 115 aa, synthetic construct
QVQLVQSGAEVKKPGSSVKVSCKASGGTFSSSWMNWVKQAPGQGLEWIGRIYREDGHTNYNGKFKGRATLTADKSTSTAYMELSSLRSEDTAVYFCANGGAMDYWGQGTTVTVSS

SEQ ID NO: 192 - protein, 115 aa, synthetic construct
QVQLVQSGAEVKKPGSSVKVSCKASGGTFSSSWMNWVKQAPGQGLEWIGRIYREDGHTNYNGKFKGRATITADKSTSTAYMELSSLRSEDTAVYFCANGGAMDYWGQGTTVTVSS

SEQ ID NO: 193 - protein, 107 aa, synthetic construct
DIQMTQSPSSLSASVGDRVTITCRASQDISNYLNWYQQKPGKVPKLLIYYTSRLHSGVPSRFSGSGSGTDFTLTISSLQPEDVATYYCQQDNTLPWTFGGGTKLEIK

SEQ ID NO: 194 - protein, 107 aa, synthetic construct
DIQMTQSPSSLSASVGDRVTITCRASQDISNYLNWYQQKPGKVPKLLIYYTSRLHSGVPSRFSGSGSGTDYTLTISSLQPEDVATYFCQQDNTLPWTFGGGTKLEIK

SEQ ID NO: 195 - protein, 115 aa, synthetic construct
QVQLVQSGAEVKKPGSSVKVSCKASGYAFSSSWMNWVRQAPGQGLEWMGRIYREDGHTNYNGKFKGRVTITADKSTTTAYMELSSLRSEDTAVYYCANGGAMDYWGQGTLVTVSS

SEQ ID NO: 196 - protein, 115 aa, synthetic construct
QVQLVQSGAEVKKPGSSVKVSCKASGGTFSSSWMNWVRQAPGQGLEWMGRIYREDGHTNYNGKFKGRVTITADKSTSTAYMELSSLRSEDTAVYYCANGGAMDYWGQGTLVTVSS

SEQ ID NO: 197 - protein, 115 aa, synthetic construct
QVQLVQSGAEVKKPGASVKVSCKASGYAFSSSWMNWVRQAPGQGLEWMGRIYREDGHTNYNGKFKGRVTMTADKSITTAYMELSRLRSDDTAVYYCANGGAMDYWGQGTLVTVSS

SEQ ID NO: 198 - protein, 115 aa, synthetic construct
QVQLVQSGAEVKKPGASVKVSCKASGYTFSSSWMNWVRQAPGQGLEWMGRIYREDGHTNYNGKFKGRVTMTADKSITTAYMELSRLRSDDTAVYYCANGGAMDYWGQGTLVTVSS

SEQ ID NO: 199 - protein, 115 aa, synthetic construct
QVQLVQSGAEVKKPGASVKVSCKASGYAFSSSWMNWVRQAPGQGLEWMGRIYREDGHTNYNGKFKGRVTMTADKSTTTAYMELSSLRSEDTAVYYCANGGAMDYWGQGTLVTVSS

SEQ ID NO: 200 - protein, 115 aa, synthetic construct
QVQLVQSGAEVKKPGASVKVSCKASGYTFSSSWMNWVRQAPGQGLEWMGRIYREDGHTNYNGKFKGRVTMTADKSTTTGYMELSSLRSEDTAVYYCANGGAMDYWGQGTLVTVSS

SEQ ID NO: 201 - protein, 115 aa, synthetic construct
QVQLVQSGAEVKKPGASVKVSCKASGYAFSSSWMNWVRQAPGQRLEWMGRIYREDGHTNYNGKFKGRVTITADKSATTAYMELSSLRSEDTAVYYCANGGAMDYWGQGTLVTVSS

SEQ ID NO: 202 - protein, 115 aa, synthetic construct
QVQLVQSGAEVKKPGASVKVSCKASGYTFSSSWMNWVRQAPGQRLEWMGRIYREDGHTNYNGKFKGRVTITADKSATTAYMELSSLRSEDTAVYYCANGGAMDYWGQGTLVTVSS

SEQ ID NO: 203 - protein, 115 aa, synthetic construct
QVQLVQSGAEVKKPGASVKVSCKASGYAFSSSWMNWVRQAPGQGLEWMGRIYREDGHTNYNGKFKGRVTMTADKSTTTAYMELRSLRSDDTAVYYCANGGAMDYWGQGTLVTVSS

SEQ ID NO: 204 - protein, 115 aa, synthetic construct
QVQLVQSGAEVKKPGASVKVSCKASGYTFSSSWMNWVRQAPGQGLEWMGRIYREDGHTNYNGKFKGRVTMTADKSTSTAYMELRSLRSDDTAVYYCANGGAMDYWGQGTLVTVSS

SEQ ID NO: 205 - protein, 107 aa, synthetic construct
DIQMTQSPSSLSASVGDRVTITCRASQDISNYLNWYQQKPGKAPKLLIYYTSRLHSGVPSRFSGSGSGTDYTFTISSLQPEDIATYFCQQDNTLPWTFGGGTKVEIK

SEQ ID NO: 206 - protein, 107 aa, synthetic construct
DIQMTQSPSSLSASVGDRVTITCRASQDISNYLNWYQQKPGKAPKLLIYYTSRLHSGVPSRFSGSGSGTDYTFTISSLQPEDIATYYCQQDNTLPWTFGGGTKVEIK

SEQ ID NO: 207 - protein, 107 aa, synthetic construct
DIQMTQSPSSLSASVGDRVTITCRASQDISNYLNWYQQKPGKAPKLLIYYTSRLHSGVPSRFSGSGSGTDYTLTISSLQPEDIATYFCQQDNTLPWTFGGGTKVEIK

SEQ ID NO: 208 - protein, 107 aa, synthetic construct
DIQMTQSPSSLSASVGDRVTITCRASQDISNYLNWYQQKPGKAPKLLIYYTSRLHSGVPSRFSGSGSGTDYTLTISSLQPEDFATYFCQQDNTLPWTFGGGTKVEIK

SEQ ID NO: 209 - protein, 107 aa, synthetic construct
EIVMTQSPATLSLSPGERATLSCRASQDISNYLNWYQQKPGQAPRLLIYYTSRLHSGIPARFSGSGSGTDYTLTISSLEPEDIAVYFCQQDNTLPWTFGGGTKVEIK

SEQ ID NO: 210 - protein, 107 aa, synthetic construct
EIVMTQSPATLSLSPGERATLSCRASQDISNYLNWYQQKPGQAPRLLIYYTSRLHSGIPARFSGSGSGTDYTLTISSLEPEDFAVYYCQQDNTLPWTFGGGTKVEIK

SEQ ID NO: 211 - protein, 107 aa, synthetic construct
DIVMTQSPDSLAVSLGERATINCRASQDISNYLNWYQQKPGQPPKLLIYYTSRLHSGVPDRFSGSGSGTDYTLTISSLQAEDIAVYFCQQDNTLPWTFGGGTKVEIK

SEQ ID NO: 212 - protein, 107 aa, synthetic construct
DIVMTQSPDSLAVSLGERATINCRASQDISNYLNWYQQKPGQPPKLLIYYTSRLHSGVPDRFSGSGSGTDYTLTISSLQAEDIAVYYCQQDNTLPWTFGGGTKVEIK

SEQ ID NO: 213 - protein, 107 aa, synthetic construct
DIQMTQSPSTLSASVGDRVTITCRASQDISNYLNWYQQKPGKAPKLLIYYTSRLHSGVPSRFSGSGSGTEYTLTISSLQPDDIATYFCQQDNTLPWTFGGGTKVEIK

SEQ ID NO: 214 - protein, 107 aa, synthetic construct
DIQMTQSPSTLSASVGDRVTITCRASQDISNYLNWYQQKPGKAPKLLIYYTSRLHSGVPSRFSGSGSGTEYTLTISSLQPDDFATYFCQQDNTLPWTFGGGTKVEIK

SEQ ID NO: 215 - protein, 122 aa, synthetic construct
EVKLVESGGGLVQPGGSLSLSCAASGFTFTDYYMSWVRQPPGKALEWLGFIRNKGNAYTTENSASVKGRFTISRDNSQSILYLQMNALRAEDSATYYCARYRGNPHYAMDYWGQGTSVTVSS

SEQ ID NO: 216 - protein, 122 aa, synthetic construct
EVQLVESGGGLVQPGGSLRLSCAASGFTFTDYYMSWVRQAPGKGLEWVGFIRNKGNGYTTENSASVKGRFTISRDNSKSTLYLQMNSLRAEDTAVYYCARYRGNPHYAMDYWGQGTLVTVSS

SEQ ID NO: 217 - protein, 122 aa, synthetic construct
EVQLVESGGGLIQPGGSLRLSCAASGFTFTDYYMSWVRQPPGKGLEWVGFIRNKGNGYTTENSASVKGRFTISRDNSKSTLYLQMNSLRAEDTAVYYCARYRGNPHYAMDYWGQGTLVTVSS

SEQ ID NO: 218 - protein, 122 aa, synthetic construct
QVQLVESGGGVVQPGGSLRLSCAASGFTFTDYYMSWVRQAPGKGLEWVGFIRNKGNGYTTENSASVKGRFTISRDNSKSTLYLQMNSLRAEDTAVYYCARYRGNPHYAMDYWGQGTLVTVSS

SEQ ID NO: 219 - protein, 122 aa, synthetic construct
EVQLVESGGGLVQPGGSLRLSCAASGFTFTDYYMSWVRQAPGKGLEWVGFIRNKGNGYTTENSASVKGRFTISRDNSKSSLYLQMNSLKTEDTAVYYCARYRGNPHYAMDYWGQGTLVTVSS

SEQ ID NO: 220 - protein, 122 aa, synthetic construct
EVQLVESGGGLVQPGRSLRLSCTASGFTFTDYYMSWVRQAPGKGLEWVGFIRNKGNGYTTENSASVKGRFTISRDNSKSILYLQMNSLKTEDTAVYYCARYRGNPHYAMDYWGQGTLVTVSS

SEQ ID NO: 221 - protein, 122 aa, synthetic construct
EVQLVESGGGLVQPGGSLRLSCAASGFTFTDYYMSWVRQAPGKGLEWVGFIRNKGNGYTTENSASVKGRFTISRDNAKSSLYLQMNSLRAEDTAVYYCARYRGNPHYAMDYWGQGTLVTVSS

SEQ ID NO: 222 - protein, 111 aa, synthetic construct
DIVLTQSPDSLAVSLGERATINCRASESVEFYGTSFLQWYQQKPGQPPKLLIYGASNVESGVPDRFSGSGSGTDFTLTISSLQAEDIAVYFCQQSRKVPSTFGGGTKVEIK

SEQ ID NO: 223 - protein, 111 aa, synthetic construct
EIVLTQSPATLSVSPGERATLSCRASESVEFYGTSFLQWYQQKPGQAPRLLIYGASNVESGIPARFSGSGSGTEFTLTISSLQSEDIAVYFCQQSRKVPSTFGGGTKVEIK

SEQ ID NO: 224 - protein, 111 aa, synthetic construct
DIQLTQSPSSLSASVGDRVTITCRASESVEFYGTSFLQWYQQKPGKAPKLLIYGASNVESGVPSRFSGSGSGTDFTLTISSLQPEDIATYFCQQSRKVPSTFGGGTKVEIK

SEQ ID NO: 225 - protein, 111 aa, synthetic construct
DIVLTQSPLSLPVTPGEPASISCRASESVEFYGTSFLQWYLQKPGQSPQLLIYGASNVESGVPDRFSGSGSGTDFTLKISRVEAEDIGVYFCQQSRKVPSTFGGGTKVEIK

SEQ ID NO: 226 - protein, 111 aa, synthetic construct
EIVLTQSPGTLSLSPGERATLSCRASESVEFYGTSFLQWYQQKPGQAPRLLIYGASNVESGIPDRFSGSGSGTDFTLTISRLEPEDIAVYFCQQSRKVPSTFGGGTKVEIK

SEQ ID NO: 227 - protein, 120 aa, synthetic construct
DVQLVESGGGLVQPGGSRKLSCTASGFTFSNFGMHWVRQAPETGLEWVAYISSGSSTFYYADAVKGRFTISRDNPKNTLFLQMTSLRSEDTAMYFCARSPAYYRYGLDYWGQGTTLTVSS

SEQ ID NO: 228 - protein, 120 aa, synthetic construct
EVQLVESGGGVVQPGRSLRLSCAASGFTFSNFGMHWVRQAPGKGLEWVAYISSGSSTFYYADSVKGRFTISRDNSKNTLYLQMNSLRAEDTAVYYCARSPAYYRYGLDYWGQGTTVTVSS

SEQ ID NO: 229 - protein, 120 aa, synthetic construct
EVQLVESGGGVVQPGRSLRLSCAASGFTFSNFGMHWVRQAPGKGLEWVAYISSGSSTFYYADSVKGRFTISRDNSKNTLYLQMNSLRAEDTAVYFCARSPAYYRYGLDYWGQGTTVTVSS

SEQ ID NO: 230 - protein, 111 aa, synthetic construct
DIVMTQTPLSLSVTPGQPASISCRASQSVSSSTFSYMHWYQQKPGQPPQLLIYSSSNLESGVPDRFSGSGSGTDFTLKISRVEAEDVGVYYCQHSWEIPYTFGGGTKVEIK

SEQ ID NO: 231 - protein, 111 aa, synthetic construct
DIVMTQTPLSLSVTPGQPASISCRASQSVSSSTFSYMHWYQQKPGQPPQLLIKSSSNLESGVPDRFSGSGSGTDFTLKISRVEAEDVGVYYCQHSWEIPYTFGGGTKVEIK

SEQ ID NO: 232 - protein, 111 aa, synthetic construct
DIVLTQTPLSLSVTPGQPASISCRASQSVSSSTFSYMHWYQQKPGQPPQLLIKSSSNLESGVPDRFSGSGSGTDFTLKISRVEAEDVGVYYCQHSWEIPYTFGGGTKVEIK

SEQ ID NO: 233 - protein, 111 aa, synthetic construct
DIVMTQSPDSLAVSLGERATINCRASQSVSSSTFSYMHWYQQKPGQPPKLLIYSSSNLESGVPDRFSGSGSGTDFTLTISSLQAEDVAVYYCQHSWEIPYTFGGGTKVEIK

SEQ ID NO: 234 - protein, 111 aa, synthetic construct
DIVMTQSPDSLAVSLGERATINCRASQSVSSSTFSYMHWYQQKPGQPPKLLIKSSSNLESGVPDRFSGSGSGTDFTLTISSLQAEDVAVYYCQHSWEIPYTFGGGTKVEIK

SEQ ID NO: 235 - protein, 111 aa, synthetic construct
DIVLTQSPDSLAVSLGERATINCRASQSVSSSTFSYMHWYQQKPGQPPKLLIKSSSNLESGVPDRFSGSGSGTDFTLTISSLQAEDVAVYYCQHSWEIPYTFGGGTKVEIK

SEQ ID NO: 236 - protein, 118 aa, synthetic construct
DVQLHESGPGLVKPSQSLSLTCSVTGYSITNNYYWNWIRQFPGNNLEWMGYITYDASNNYNPSLKNRISVTRDTSKNQFFLKLSSVTTEDTATYYCTRGGGQLRFDYWGQGTTLTVSS

SEQ ID NO: 237 - protein, 118 aa, synthetic construct
EVQLQESGPGLVKPSDTLSLTCAVSGYSISNNYYWNWIRQPPGKGLEWIGYITYDGSNNYNPSLKNRVTMSVDTSKNQFSLKLSSVTAVDTAVYYCARGGGQLRFDYWGQGTTVTVSS

SEQ ID NO: 238 - protein, 118 aa, synthetic construct
EVQLQESGPGLVKPSDTLSLTCAVSGYSISNNYYWNWIRQPPGKGLEWIGYITYDGSNNYNPSLKNRVTMSRDTSKNQFSLKLSSVTAVDTAVYYCARGGGQLRFDYWGQGTTVTVSS

SEQ ID NO: 239 - protein, 118 aa, synthetic construct
EVQLQESGPGLVKPSDTLSLTCAVSGYSISNNYYWNWIRQPPGKGLEWIGYITYDGSNNYNPSLKNRITMSRDTSKNQFSLKLSSVTAVDTAVYYCARGGGQLRFDYWGQGTTVTVSS

SEQ ID NO: 240 - protein, 118 aa, synthetic construct
EVQLQESGPGLVKPSDTLSLTCAVSGYSISNNYYWNWIRQPPGKGLEWMGYITYDGSNNYNPSLKNRITVSRDTSKNQFSLKLSSVTAVDTAVYYCARGGGQLRFDYWGQGTTVTVSS

SEQ ID NO: 241 - protein, 118 aa, synthetic construct
EVQLQESGPGLVKPSDTLSLTCAVSGYSITNNYYWNWIRQPPGKGLEWMGYITYDGSNNYNPSLKNRITVSRDTSKNQFSLKLSSVTAVDTAVYYCTRGGGQLRFDYWGQGTTVTVSS

SEQ ID NO: 242 - protein, 107 aa, synthetic construct
DIQMTQSPSSLSASVGDRVTITCKASQSVSNEVTWYQQKPGKAPKLLIYYASNRYTGVPSRFSGSGSGTDFTFTISSLQPEDIATYYCQQDYSSPWTFGGGTKVEIK

SEQ ID NO: 243 - protein, 107 aa, synthetic construct
DIQMTQSPSSLSASVGDRVTITCKASQSVSNEVTWYQQKPGKAPKLLIYYASNRYTGVPDRFSGSGSGTDFTFTISSLQPEDIATYYCQQDYSSPWTFGGGTKVEIK

SEQ ID NO: 244 - protein, 107 aa, synthetic construct
DIQMTQSPSSLSASVGDRVTITCKASQSVSNEVTWYQQKPGKAPKMLIYYASNRYTGVPDRFSGSGSGTDFTFTISSLQPEDIATYYCQQDYSSPWTFGGGTKVEIK

SEQ ID NO: 245 - protein, 107 aa, synthetic construct
DIQMTQSPSSLSASVGDRVTITCKASQSVSNEVTWYQQKPGKAPKMLIYYASNRYTGVPDRFSGSGYGTDFTFTISSLQPEDIATYYCQQDYSSPWTFGGGTKVEIK

SEQ ID NO: 246 - protein, 107 aa, synthetic construct
DIQMTQSPSSLSASVGDRVTITCKASQSVSNEVTWYQQKPGKSPKMLIYYASNRYTGVPDRFSGSGYGTDFTFTISSLQPEDIATYFCQQDYSSPWTFGGGTKVEIK

SEQ ID NO: 247 - protein, 107 aa, synthetic construct
SIVMTQSPSSLSASVGDRVTITCKASQSVSNEVTWYQQKPGKSPKMLIYYASNRYTGVPDRFSGSGYGTDFTFTISSLQPEDIATYFCQQDYSSPWTFGGGTKVEIK

SEQ ID NO: 248 - protein, 122 aa, synthetic construct
EVQLVESGGGLVQPGGSLRLSCAASGFTFTDYYMSWVRQAPGKGLEWVGFIRNKGNAYTTENSASVKGRFTISRDNSKSSLYLQMNSLKTEDTAVYYCARYRGNPHYAMDYWGQGTLVTVSS

SEQ ID NO: 249 - protein, 122 aa, synthetic construct
EVQLVESGGGLVQPGGSLRLSCAASGFTFTDYYMSWVRQAPGKGLEWVGFIRNKGNGYTTEYSASVKGRFTISRDNSKSSLYLQMNSLKTEDTAVYYCARYRGNPHYAMDYWGQGTLVTVSS

SEQ ID NO: 250 - protein, 122 aa, synthetic construct
EVQLVESGGGLVQPGGSLRLSCAASGFTFTDYYMSWVRQAPGKGLEWVGFIRNKGNAYTTEYSASVKGRFTISRDNSKSSLYLQMNSLKTEDTAVYYCARYRGNPHYAMDYWGQGTLVTVSS

SEQ ID NO: 251 - protein, 122 aa, synthetic construct
EVQLVESGGGLVQPGRSLRLSCTASGFTFTDYYMSWVRQAPGKGLEWVGFIRNKGNAYTTENSASVKGRFTISRDNSKSILYLQMNSLKTEDTAVYYCARYRGNPHYAMDYWGQGTLVTVSS

SEQ ID NO: 252 - protein, 122 aa, synthetic construct
EVQLVESGGGLVQPGRSLRLSCTASGFTFTDYYMSWVRQAPGKGLEWVGFIRNKGNGYTTEYSASVKGRFTISRDNSKSILYLQMNSLKTEDTAVYYCARYRGNPHYAMDYWGQGTLVTVSS

SEQ ID NO: 253 - protein, 122 aa, synthetic construct
EVQLVESGGGLVQPGRSLRLSCTASGFTFTDYYMSWVRQAPGKGLEWVGFIRNKGNAYTTEYSASVKGRFTISRDNSKSILYLQMNSLKTEDTAVYYCARYRGNPHYAMDYWGQGTLVTVSS

SEQ ID NO: 254 - protein, 122 aa, synthetic construct
EVQLVESGGGLVQPGGSLRLSCAASGFTFTDYYMSWVRQAPGKGLEWVGFIRNKGNAYTTENSASVKGRFTISRDNAKSSLYLQMNSLRAEDTAVYYCARYRGNPHYAMDYWGQGTLVTVSS

SEQ ID NO: 255 - protein, 122 aa, synthetic construct
EVQLVESGGGLVQPGGSLRLSCAASGFTFTDYYMSWVRQAPGKGLEWVGFIRNKGNGYTTEYSASVKGRFTISRDNAKSSLYLQMNSLRAEDTAVYYCARYRGNPHYAMDYWGQGTLVTVSS

SEQ ID NO: 256 - protein, 122 aa, synthetic construct
EVQLVESGGGLVQPGGSLRLSCAASGFTFTDYYMSWVRQAPGKGLEWVGFIRNKGNAYTTEYSASVKGRFTISRDNAKSSLYLQMNSLRAEDTAVYYCARYRGNPHYAMDYWGQGTLVTVSS

SEQ ID NO: 257 - protein, 120 aa, synthetic construct
EVQLVESGGGVVQPGRSLRLSCAASGFTFSNFGMHWVRQAPGKGLEWVAYISSGSSTFYYADAVKGRFTISRDNSKNTLYLQMNSLRAEDTAVYYCARSPAYYRYGLDYWGQGTTVTVSS

SEQ ID NO: 258 - protein, 111 aa, synthetic construct; identical to SEQ ID NO: 231

SEQ ID NO: 259 - protein, 118 aa, synthetic construct
EVQLQESGPGLVKPSDTLSLTCAVSGYSISNNYYWNWIRQPPGKGLEWIGYITYDASNNYNPSLKNRVTMSRDTSKNQFSLKLSSVTAVDTAVYYCARGGGQLRFDYWGQGTTVTVSS

SEQ ID NO: 260 - protein, 118 aa, synthetic construct
EVQLQESGPGLVKPSDTLSLTCAVSGYSISNNYYWNWIRQPPGKGLEWIGYITYDASNNYNPSLKNRITMSRDTSKNQFSLKLSSVTAVDTAVYYCARGGGQLRFDYWGQGTTVTVSS

SEQ ID NO: 261 - protein, 118 aa, synthetic construct
EVQLQESGPGLVKPSDTLSLTCAVSGYSISNNYYWNWIRQPPGKGLEWMGYITYDASNNYNPSLKNRITVSRDTSKNQFSLKLSSVTAVDTAVYYCARGGGQLRFDYWGQGTTVTVSS

SEQ ID NO: 262 - protein, 107 aa, synthetic construct
DIQMTQSPSSLSASVGDRVTITCRASQDISNYLNWYQQKPGKAPKLLIYYTSRLHSGVPSRFSGSGSGTDYTFTISSLQPEDIATYFCGNDNTLPWTFGGGTKVEIK

SEQ ID NO: 263 - protein, 107 aa, synthetic construct
DIQMTQSPSSLSASVGDRVTITCRASQDISNYLNWYQQKPGKAPKLLIYYTSRLHSGVPSRFSGSGSGTDYTFTISSLQPEDIATYFCANDNTLPWTFGGGTKVEIK

SEQ ID NO: 264 - protein, 9 aa, synthetic construct
GNDNTLPWT

SEQ ID NO: 265 - protein, 9 aa, synthetic construct
ANDNTLPWT

SEQ ID NO: 266 - protein, 19 aa, synthetic construct
FIRNKGNAYTTENSASVKG

SEQ ID NO: 267 - protein, 19 aa, synthetic construct
FIRNKGNGYTTEYSASVKG